European Patent Specification EP 3 719 039 B1, published July 26, 2023. Title: BINDING MOLECULES SPECIFIC FOR ASCT2 AND USES THEREOF. Applicant: MEDIMMUNE, LLC. Application PCT/US2016/061219. The sequence listing filed with the application follows.

SEQUENCE LISTING (27 sequences)

SEQ ID NO: 1 - protein, 122 aa, Artificial Sequence
  source: /note="Description of Artificial Sequence: Synthetic polypeptide"
QVQLQQWGAGLLKPSETLSLTCAVYGGSFSGYYWSWIRQPPGKGLEWIGEIHHSGGANYNPSLKSRVTISVDTSKNQFSLKLTSVTAADTAVYYCARGQGKNWHYDYFDYWGQGTLVTVSSA

SEQ ID NO: 2 - protein, 107 aa, Artificial Sequence
  source: /note="Description of Artificial Sequence: Synthetic polypeptide"
DIQMTQSPSTLSTSVGDRVTLTCRASQSIRSWLAWYQQNPGKAPKLLIYKASILKIGVPSRFSGSGSGTDFTLTITSLQPDDFATYYCQQYYSYSRTFGQGTKVEIK

SEQ ID NO: 3 - protein, 122 aa, Artificial Sequence
  source: /note="Description of Artificial Sequence: Synthetic polypeptide"
QVQLQQWGAGLLKPSETLSLTCAVYGGSFSGYYWSWIPQPPGKGVEWIGEINHSGSTNYNPSLKSRVTISSDTSKNQFSLKLTSVTAADTAVYYCARGQGKNWNYDYFDYWGQGTLVTVSSA

SEQ ID NO: 4 - protein, 107 aa, Artificial Sequence
  source: /note="Description of Artificial Sequence: Synthetic polypeptide"
DIQMTQSPSTLSASVGDRVTLTCRASQSIRSWLAWYQQKPGKAPKLLIYKASSLKSGVPSRFSGSGSGTDFTLTISSLQPDDFATYYCQQYYSFSRTFGQGTKVEIK

SEQ ID NO: 5 - protein, 122 aa, Artificial Sequence
  source: /note="Description of Artificial Sequence: Synthetic polypeptide"
QVQLQQWGAGLLKPSETLSLTCAVYGGSFSGYYWSWIRQPPGKGLEWIGEIHHSGGANYNPSLKSRVTISVDTSKNQFSLKLSSVTAADTAVYYCARGQGKNWHYDYFDYWGQGTLVTVSSA

SEQ ID NO: 6 - protein, 107 aa, Artificial Sequence
  source: /note="Description of Artificial Sequence: Synthetic polypeptide"
DIQMTQSPSTLSASVGDRVTITCRASQSIRSWLAWYQQKPGKAPKLLIYKASILKIGVPSRFSGSGSGTEFTLTISSLQPDDFATYYCQQYYSYSRTFGQGTKVEIK

SEQ ID NO: 7 - protein, 122 aa, Artificial Sequence
  source: /note="Description of Artificial Sequence: Synthetic polypeptide"
QVQLQQWGAGLLKPSETLSLTCAVYGGSFSGYYWSWIRQPPGKGLEWIGEIHHSGSTNYNPSLKSRVTISVDTSKNQFSLKLSSVTAADTAVYYCARGQGKNWNYDYFDYWGQGTLVTVSSA

SEQ ID NO: 8 - protein, 107 aa, Artificial Sequence
  source: /note="Description of Artificial Sequence: Synthetic polypeptide"
DIQMTQSPSTLSASVGDRVTITCRASQSIRSWLAWYQQKPGKAPKLLIYKASSLKSGVPSRFSGSGSGTEFTLTISSLQPDDFATYYCQQYYSFSRTFGQGTKVEIK

SEQ ID NO: 9 - protein, 330 aa, Artificial Sequence
  source: /note="Description of Artificial Sequence: Synthetic polypeptide"
STKGPSVFPLAPSSKSTSGGTAALGCLVKDYFPEPVTVSWNSGALTSGVHTFPAVLQSSGLYSLSSVVTVPSSSLGTQTYICNVNHKPSNTKVDKRVEPKSCDKTHTCPPCPAPELLGGPSCVFLFPPKPKDTLMISRTPEVTCVVVDVSHEDPEVKFNWYVDGVEVHNAKTKPREEQYNSTYRVVSVLTVLHQDWLNGKEYKCKVSNKALPAPIEKTISKAKGQPREPQVYTLPPSREEMTKNQVSLTCLVKGFYPSDIAVEWESNGQPENNYKTTPPVLDSDGSFFLYSKLTVDKSRWQQGNVFSCSVMHEALHNHYTQKSLSLSPGK

SEQ ID NO: 10 - protein, 5 aa, Artificial Sequence
  source: /note="Description of Artificial Sequence: Synthetic peptide"
GYYWS

SEQ ID NO: 11 - protein, 16 aa, Artificial Sequence
  source: /note="Description of Artificial Sequence: Synthetic peptide"
EIHHSGGANYNPSLKS

SEQ ID NO: 12 - protein, 13 aa, Artificial Sequence
  source: /note="Description of Artificial Sequence: Synthetic peptide"
GQGKNWHYDYFDY

SEQ ID NO: 13 - protein, 11 aa, Artificial Sequence
  source: /note="Description of Artificial Sequence: Synthetic peptide"
RASQSIRSWLA

SEQ ID NO: 14 - protein, 7 aa, Artificial Sequence
  source: /note="Description of Artificial Sequence: Synthetic peptide"
KASILKI

SEQ ID NO: 15 - protein, 9 aa, Artificial Sequence
  source: /note="Description of Artificial Sequence: Synthetic peptide"
QQYYSYSRT

SEQ ID NO: 16 - protein, 5 aa, Artificial Sequence
  source: /note="Description of Artificial Sequence: Synthetic peptide"
GYYWS

SEQ ID NO: 17 - protein, 16 aa, Artificial Sequence
  source: /note="Description of Artificial Sequence: Synthetic peptide"
EIHHSGSTNYNPSLKS

SEQ ID NO: 18 - protein, 13 aa, Artificial Sequence
  source: /note="Description of Artificial Sequence: Synthetic peptide"
GQGKNWNYDYFDY

SEQ ID NO: 19 - protein, 11 aa, Artificial Sequence
  source: /note="Description of Artificial Sequence: Synthetic peptide"
RASQSIRSWLA

SEQ ID NO: 20 - protein, 7 aa, Artificial Sequence
  source: /note="Description of Artificial Sequence: Synthetic peptide"
KASSLKS

SEQ ID NO: 21 - protein, 9 aa, Artificial Sequence
  source: /note="Description of Artificial Sequence: Synthetic peptide"
QQYYSFSRT

SEQ ID NO: 22 - protein, 16 aa, Artificial Sequence
  source: /note="Description of Artificial Sequence: Synthetic peptide"
  VARIANT (7)..(7): /replace="Gly"
  VARIANT (8)..(8): /replace="Thr"
  MISC_FEATURE (1)..(9): /note="Variant residues given in the sequence have no preference with respect to those in the annotations for variant positions"
EIHHSGSANYNPSLKS

SEQ ID NO: 23 - protein, 13 aa, Artificial Sequence
  source: /note="Description of Artificial Sequence: Synthetic peptide"
  VARIANT (7)..(7): /replace="Asn"
  MISC_FEATURE (1)..(9): /note="Variant residues given in the sequence have no preference with respect to those in the annotations for variant positions"
GQGKNWHYDYFDY

SEQ ID NO: 24 - protein, 7 aa, Artificial Sequence
  source: /note="Description of Artificial Sequence: Synthetic peptide"
  VARIANT (4)..(4): /replace="Ser"
  VARIANT (7)..(7): /replace="Ser"
  MISC_FEATURE (1)..(9): /note="Variant residues given in the sequence have no preference with respect to those in the annotations for variant positions"
KASILKI

SEQ ID NO: 25 - protein, 9 aa, Artificial Sequence
  source: /note="Description of Artificial Sequence: Synthetic peptide"
  VARIANT (6)..(6): /replace="Phe"
  MISC_FEATURE (1)..(9): /note="Variant residues given in the sequence have no preference with respect to those in the annotations for variant positions"
QQYYSYSRT

SEQ ID NO: 26 - protein, 107 aa, Homo sapiens [sequence omitted]

SEQ ID NO: 27 - protein, 6 aa, Artificial Sequence
  source: /note="Description of Artificial Sequence: Synthetic 6xHis tag"
HHHHHH